European Patent Specification EP 4 580 655 B1, published September 9, 2026. Title: Lyofilizované tablety s antimikrobiálním účinkem proti bakteriím Staphylococcus aureus a Pseudomonas aeruginosa s obsahem bakteriofágů a lytických enzymů s optimální stabilitou a efektivitou aktivních složek. Applicant: MB PHARMA s.r.o. The sequence listing filed with the application follows.

SEQUENCE LISTING (3 sequences)

SEQ ID NO: 1 - protein, 259 aa, Bacteriophage Staphylococcus sciuri S10
METLKDAENYIKKAIGKGIDFDGQYGYQCADLSVDYMYYITDKKVRMWGNAKDLINNDFKGLATVYKNTPSFLAKKGDVFVMGANRGGGYGHTGIVTSATLNSITVIEQNWLGGGATFSEVTTKRTHPYDTEMWFIRPKFAKSKTKETAKKVAKASAKKVTPKKSWSFKVGGEPIITRIGKPSLKATSGGSVKPNQKMTFNKLVKSEGYEWGKLTNYKGQTEYVPIRPLKQKGYWGVLKWNSSSVDKLAAALEHHHHHH

SEQ ID NO: 2 - DNA, 17847 bp, Bacteriophage Staphylococcus aureus DSM 34647
  source 1..17847: mol_type = genomic DNA
tttatgtatctattgacttttattcaaagttatgatttgaaattaaaatcttatttcttctattaaatagtatttataaaattatttaaactttttaagaaaaactgttgacaaaacttttaaatgtttgctatactatgtatgtaatcaaacaaggaggtaacaaaatggaaaatgaaacaaaaaacattgagttgaagcatgtttttcgttttaagaatggaaatttatgtatagcgttatttgatagaacagaaaatgaaatttcattttatgatgttgacattgatgaaattgaagatttaaatcataattctgttttacgtgtaatttcaactttattaggatgtgataataatgattaatgttgataatgcaccagaagaaaaaggacaagcctacactgaaatgttgcaactattcaataaaatgattcaatggaatccagcttatacatttgacaatgcaattaacttagtagcagcttgccaacaactattattaaactataacagttctgttgttcaattcttaaaagatgaactaaacaatgaaattaaaccagaatcaatattatcttacattgctggtgatgacccaatagaacaatggaatatgcacaaaggattttatgaaacgtataacgtttacgttttttagaaaggagtgatataataatgaaacctgatgatattgttacattacgaattaaaggttatattcttcactatttagatgataaaaatgaatatgttgaagaatttataccacttcatgagtatcatttatcaaaaacacaagcaaaagacttattacctaattcacacaaacttttatccactacacgcacaacgaaaacaattcaagtttattacaatgatttaataaaaatcgcaattccagaaagcaaataatttaaataagaggagacataaaaatgacaaacgtaaaagatattttatcaagacaccaaaacacattagcgagattcgaatttgaggaaaaagaaagagaatttatcaaactttcagaacttgtagaaaaatatggaataaaaaaagaatacatcgttagagcattattcacaaacaaagaatcaaaattcggtgtacaaggtgttatcgtcactgacgactataatgtaaacttaccgaaccacttaacagagttaattaaaaaaatgagagcagatgaggacgttgttaacattatcaatgctggtgaagtgcaatttacaatttatgaatatgaaaacaaaaaaggtcaaaaaggttactcaatcaactttggtcaagtatcattttaatacaatttcataggggatatttatcccctatttttatgaggtgctaaacaatggaaaaaatatacactgccgtattattatacaatgtatcaattaatgaaacatatgaacatgaaattgaacaattcgaaaaaataaataaagttaaggtaatatatagttattttgacgcaaacttttacaaaaaaggtgcatataatctttgtgtaaaatacattaaggagatataaaatgaaaattaaaaaaatttttaaattattagatttactttgttacattgatgataatagagaaaaatttaaagacaaaaaaatacaatttatttctgatagtggttttaattttgttggtattgattctgataatgatattactatcaatttttctgaagctcataataacgatttaacaatgaataatgatttattcactttagacgctgacattaatattcatactcatcgttttgattttcttaaagttatttatggaaaattttcaaataaaaattatagaaaagaaatatttacaggttgcactattgatgatgtattaaaatatttcgagaatctattatatgatgatattataataatttaccaaaacaaagttatatacgataacgggaaagtgatagaccatgaataatatactggatattattattgttttccttttagcatttttaattacacttgtaatacttatgacaatgcatatacgtgtgtcatttggtgttttatttactacattgattatattctacattatctttttagtggttatatatggtttatatggaggtcgttagcaatggttagacatacgtccgaaatggataaatggaaaaaagaaagagacgcaagaaaagagcaggaaaaagaattgtttttaaatgattttagtactgttaattttaaatttgatgataaagatttacaagaggcgtacatagacgcatggaaacatttcgcacatttgccctattttccaaaagaaagacacgtgtcacatgcaaatgctgtatcattggtaagaggtaaaagacatgaacaattaaactatatacttgaaatatataaccgtaaagatgaatctaataataaaaacgctaaaaaacataaatatgctttatatgaattacaagcaaaaaataataattcttctatgtataaatatataaaggaaattgacactttatacaaagaaattggtaaatcagatagaccagtgactactattgatgatgaagatgtgaggtataactttttatattatgcaacatttgaagactaattttaatactgtaaacgacataataaactattacaaggagcaaaaacatggtgaaacaaaatcgtttagacatggtaagagattatcaaaatgcggtcaatcatgtaaggaaaaaaataccagaaaactataatcaaatagaattagttgatgaactcatgaatgatgatatagactattatatatctatttcaaaccgttctgacggaaaatcgttcaactatgtttcattctttatttatttagctataaaacttgatattaaatttactttattatcacgtcattatacattacgtgacgcttatcgtgattttattgaggaaatcatagacaaaaacccactattcaaatctaagcgtgtcacattcagaagcgctagggactatttagctattatttatcaagataaagaaatcggtgtgattacagatttgaatagcgctactgatttaaaatatcattctaactttttaaaacactaccctattattatatatgatgaattcttagcgcttgaagatgactatttaattgatgagtgggataagttaaaaacaatttatgaatcaatcgaccgtaaccatggtaatgttgattatattggttttcctaaaatgtttttactaggtaatgctgtcaacttttcaagtcctatattatccaatttaaatatttataatttattacaaaaacataaaatgaatacatcaagactttacaaaaacatttttttagaaatgcgtcgaaacgattacgtcaatgaaaagcgtaatacacgtgcgtttaattcaaatgatgacgctatgacaactggcgagtttgaatttaacgaatataatttggcagatgataatttaagaaatcatattaaccaaaacggtgattttttctatattaaaactgacgataaatatataaaaattatgtataatgttgatacatttaatgctaacatcattgttataccttatacaaaacaatatgagttttgtactaaaatcaaagatatagacgacaatgttatttatctaagagaagatatgttttataaagaaaacatggaacgttattattacaatccaagcaatttacattttgacaatgcatattcgaaaaattacgtggttgataatgatagatatttatatttagacatgaataaaattataaaatttcatataaaaaatgaaatgaagaaaaacatcaacgaatttgaaagaaaagaaaaaatatatgaagataactatatagaaaatacaaagaagtatttaatgaaacaatacggtttataaaaggtgtgtaagattatgggattacttgagtgtatgaaatatcataaaaatcaaagcaaaatgatattgtattgggatattgaaacattatcatacaataaaataaacggacgtaataaacctacgctatataaaaacgtaacgtattctgttgcgattggttggtttaatggttacgaaattgatgttgaagtattccctagttttgaagccttttatgatgatttttacaagtatgttaaccgtcgtgatacaatcacaaaatcaaaaacagatattattatgattgcacataactgtaataagtacgacaatcattttttacttaaagacactatgcgttattttgataatatcacacgtgaaaatatatatttaaaatctgcagaagaaaatgaacacacactaaaaatgcaagaggctactattttagcaaaaaatcaaaatgtgattttagaaaaacgtgtaaaatcctctattaatttagatttaacaatgtttttaaacggatttaaatttaatattatcgataattttatgaaaaccaatacatcaattgcgacattaggtaagaaattacttgatggtggttatttaacagaaaaccaacttaaaacagattttaattatacgatttttgataaagataatgatatgaatgatagtgaagcctatgactatgctgtaaagtgtttcgctaaactcacacctgatcaacttacatacattcataatgacgtgattatattaggtatgtgtcatattcattatagtgatatattcccaaattttgactataacaaattaacattctcattgaatattatggaatcttatttgaataatgatatgacacgttttcagttacttaatcaatatcaagatattaaaatatcttatacacattatcatttccatgatatgaatttttatgactatattaaatcattctatcgtggtggtttaaatatgtataacaccaaatacatcaataaacttattgatgagccatgtttttctatagacatcaattcgagttatccttatgtgatgtatcatgagaaaattccgacgtggttatacttttatgaacactattcagaaccaacgttaatccctacttttttagatgatgacaattatttttcattatataagattgataaagatgtatttaacgatgatttattaattaaaattaaatcacgtgtattacgtcaaatgattgtaaaatactataataacgataatgattacgttaatatcaatacaaatacattaagaatgattcaagacattacgggtattgattgcacacatatacgtgtcaattcgtttgtaatatatgaatgtgaatactttcatgcacgtgatattatttttcaaaattattttattaaaacacaaggtaagttaaaaaataaaatcaatatgacatcaccttacgactatcatatcactgatgacatcaacgaacacccatactcaaatgaggaggttatgttgtcaaaagtggtactcaatggtttatatggtatacctgctttacgttcacattttaacttatttcgtttagatgataacaatgcactatacaatatcattaacggttataaaaacactgaacgtaatattttattctctacatttgttacatcacgttcattgtataacttattggtacctttccaatacttaacggaaaatgaaattgacgacaattttatttattgtgacactgatagtttgtatatgaaatccgttgttaaacccttattgaaccccagtttattcgacccgatagccttaggtaaatgggatattgaaaacgaacagatagataagatgtttgtactgaatcataagaaatatgcatatgaagtgaatggaaagattaaaattgcttctgctggtataccgaaaaacgcctttgatacaagcgtcgattttgaaacctttgtacgtgaacaattctttgacggtgccattatagaaaacaataaaagtatctataatgaacagggtacaatatcgatatatccgtctaaaactgaaattgtatgtggtaatgtatatgatgaatattttactgatgaacttaatatgaaacgtgaatttatattaaaagacgctagagaaaatttcgatcatagtcaatttgatgatattctttatattgaaagtgacatcggttcattttcacttaacgacttatttccagttgaacgttcagtacataataaatcaaatttaaatatattaaaaaatcaacatgatgacatcaaaaaaggcaactgttaaataacagtcgcctttttcttttgagataacatgaaaaatgtgtacgaaaattgattatgttttgtattttatttactagcattactagcatgtgttcattatagcataattctttacgcaataccactgaagaatacaatattatcaccagcgttttctggtacaccattaatgagtgtatacaacaccacacgtgacggcgcaacgtaaggtggtacattatagtttgcaactaaaaacgaaccatcgtcaaatacagcaacaacaacaccagtgtgaccaataccatatgcagttgcttgtaagtatggtggtttactagaaaaaccataccctactgttggattatgtgttgtttttgcacctaactttttatagacgtaccatacacgttgaccgtttgtgatttggccgtcgtcggtaggttgtctttttccatgtagttgtgacatatacgcccatgttaattctgtacactgaccagcattaccagtttgaggaaatatgttacctggtttgtataaatattcttttttgaataaaggtacaccaattgcttttttatatttttctggtaactgtgcgtacgtccagttaccaccaatcacacgaccactttttccatttggtttgactgatttaccactaattggtttatgatctccgtcatcatcagtagggttagaactgctacccccgctatccacttgcacgctatcaatcaatttttttaatgaatcaagtaagccaattgtcattttaatatgatatgtgttgttgaatgttttttgtaatgtaaaataatcattactaaaaaatttatcactaccaatactgtgaacgtcccattgtaatgcgtcttgtactttttttaataattcttgcatggcttgtttagctaaagcgagtagtgaactaccactgtcaccactactaccactgtcagacgtgtcactaggtgaaccacctttaccgtctaatttaccaccccatgctaaaatagtatttgcaccgtctaaaaaaggattaccatagttttgtactttattatatgacgctttcaaacctaggggataatatgcagcccaagtagccgctgctgttaatggaatatatgcacgtccaattgtacctgctttcatatttttagcaaaatctgcattaccctttctttgtacgtcttgaggtacaaagtggacaatgttacctgcgtcataccaagacggttgtccagcttgttttgattgtgatactaactttcttgcaataaatttagcgtctgttaaataatcaccacgtgcagacgtatgatttaaccaacctaaaccggcactatacccctcatttttttcatatacagcaaaaagagtaggtgacacacctatctcttttactgcttttaatacttgtctgattttactttcattaccacctagccatacattaaagcgtccatacccttttactttaggcactaactggtctatcgttaaaccgaaatcatcattaatatacgaatgtgtaaatttatctatcttctcttggtcgttcattattatcactcttttcagaatcgtttttaattactcttaatttatctttaatttgttcaggcactaatacgtccatttctgcacaattttctacgatagataagccttcattagcgatataatagaaaatcgtaatcatgagtaagccaccttttaattgtaaaatctggtcaatgatgttcgctaaaatgataatacagaatatcaataattttttagcaaaacctttcattgatttttttgaccataagttattatttttaatggctttagcaaaaccagtaattacatcaacgatcattaaaacaaataaaaaatatagtaattttaaatcacctgcatatatgaacatatgaaacgcttctgtatcggtgaatcttaattttacctcattcattttatacaccctctctaaatttattatttaatggattttgtaacattggattacctgaaccgtcattatgccaaaatctcacaccggactctaaaatcgcttttaattgctccattaacatggggtcaatgtcacgtatagtatacgtacctgtacattttaaataattgcaaacagtcatactgttaattggttcaataaatgaattatagtcatttacttcaaaaccaaacaacatataatatttttgtaaaaatgtaatttcttttggtgacggtacactaattttcatcgttaaaccgttaatgctattcgcaatttggaatgcgttgcccatttctgattcagttacagacggtggttgtaaggctaaatctttatattcagcttgttgttgtttgtagaaattatattcttcattaaacttaccaaataaagcagttggacttaaattacttgctacactcacagcgtcataaaatcgtgattttgggtcactaccatttaatacattatcaatacgatttgtaattaattgactttctgcattcttttgtctattcgcttgttgtgattgtcctaagataccattattgattaatattggtacttgtgcaaaactattaaatgttatatttgtatttaagaatgaacccgtatcaatcaatatttctttatttttagcaagtatgggtctgtcgttttcagcactgttataatctactggatatactctaacttcattatgataaccaatgatcgattttgtacgtaacttaacacctgttttttgtgaaattttaccagcgtcgagtaacatcgtatttccattccaatcataaaattcaattgtcatatactcattacgtatcatatgtttaaattcatcttttttagataacatcatttcttgaagttttgtaaaacttaatgataaatcttttagactccattcttttgatttaccaccctgttttaatgtttttaatcctgtaattttttcactggtttttacgtcctctaaatcttttgtattaataaagtctttaggtaacatttgaaccttttgaaagttttgtgtaatccatggatatgcactcattttatccataaagttaataaagtcaccatattccataacgtataagttaactggtgatgtgatattgtcatatatcgtacccttagacgtgtctaagtttggctcttttttcgtaccaaatttctttgataaatcagcacttgactggaataatactatattttccaaatattgttgcatttggttatacacatagtttttattcgatacttttaacacatcgtcattattacgcaacattggtaacatatagttataggtgcgttttgataaatgttgacgttcaatattgacgtttgagagttgctctaatacattaccttgcgtgtacgtcataatagtatcaatcacaaaatatattttaaccacaacatcattcacatattcgatttgattcacaaacgcataataacgtctgtcctcaaaatctgataaaaacgtcatgtagttaatcccttgtgcgtcatgccactgcatatcaacattgatttccattctatcacgtataaaattatacggttgtttggaatagtctaacgatttaaaatgacgtccatttaaaaaataatcatcacgctctttattactattaaaatgaatcgtattttgataatcagtaaacggtgtgttatagaaaaatttaaaatttgttaattttctcatttttacctccataaaaaatagtcgtataaataatttatacgactattataacatttttattcaatgatttgtgtatctattgcaaaacgtttatcaccatttgttaagtcactatcgctataatttgatgtaacaaaatgtaattcattattaaagtttaaatataatcttgtattcatcattttattatcaatcgcacattgtgtgtagtgatgtgttgattttaagtttgcgttaatcgtacctaatttaatatcaccgtttttcttaatcccttttaatactccttttaattgtatcgttttaacaccattaattgtgacaatacgatattgcggtgcgggatatccaccattgctatcacttccaactataccactttcgagcgatatatcttgccaacctgtatcattaaattgtaattttgcactgttaattttttgattaaaattttgttcaatttctgatttagattgagcaattttattatctatatttaagttattcacttttgttgataaactgttaatacttgattcgtttgttgatgttttttgttttaaatcactaatatcattatcatatttagataaatcaacgttaccgttactgttaacaactggtctatcttttaattcttgaatatctttttcaatttttgatattttatcattatttgtttttaaagtagcgatgtcagatttaattgaattaatatcctgtgtataatctttttggttaatactgtttaattttgtttctaactcttttatcttatcaagattagcatttgttttaatatcattaatggattgttctaacgattcaagtttacctgcacttgaattttgttttaacttattaatatcctcttgtatttcttgaattgtgttgtcattgttttgtttagattttaataattcaatttgtctttcaatgtcttttattttatcaatattaacactttttttaacttcagttaattctctttttaatgcgtcaatgttttcagcaccagtatttgctttaattaaattaatttcatctgtgttacgtcctacactatctttagtagcgtttaatgattgtgtaagggtttcatatttatcatcatattttaatattgatttttcaaattcatttaattgtgtttgatgttgttctaaactttcatttaatatgacatctttttcttttaatgaatcaatctcttttttattactatcaatcattggttggaatttttttatcttctctaaaaatgttgatattttttctttgttatcattaattgcaatatcatgactttctatttgaccactgtatttattaatcaatgtttttaaatcattataaaatgttaacttataataaccagtatcagtacggacataaatatgcccgtctgatgtactgattaagtcattttcttctgttaaaaaatctgctaacctgtctattgtttcaacttgtcttaaacttcttacgattctatcagccattgttcacacctcttatttgtatcgtttccaactaaattcaaagaaaaagcctaaaatacccattatgagaacaccccccacggtacaccaacactgtaactattacctgttttaccattccattgccttactggtaaataataacgtgtaccttgccaattataaccaatccatacgtaaccatctgataaacaaatttcgtcatatggtgtataaccatttggttggaaccaatagccattaggttctgataattttggactgccgacacgtgcaaatattggtaaaaatccacatgtaaatgttccattctcatttctgtaatacgtaccatattggttttgtttccaatttccaaatgtattgaccattgatgtttctaattttttactattactacctgaaaattttggacgaataaagtgtgttacaccgtcataataatgtgttctgatggttgctttttcccaaccgtcaaaaccaccatttaaccagttttgctctaaacatgtataataatctaaatttccacttatcacacattgaatatgaccatattgagaattagtataaacagcaacgtctcctaattgtggtttaaagctcggtgtatttttatacaccgttgctaaacctttaaagtcattattaatagcgtctttggcattgccccacatacgaactttaccgtctgtaatgtaatatacataagcaactgctaagtccatacattgaaatccatatgcaccatcaaaatcaacacctacaccctcatgattatatatccattcttttgcttgttgttgtgatttcatttatatcactcctatttttgatgttttgctacccaaccatattcacgatgtttcgtttcagcattaacattactaaagaattctttatgcactttaacgttagcctccaacgtttgtcttacttctccaacagcgttaccacttgaaacacgtaaccatgcacccacttttttaatttcttctggtgcgtctctaaacaattccatttggttgccagtaatataatattcaccaggtgtagtaacgtaagctatccaattattatattgactcgcttctaaatattcttgatatggtgcatctgttttgattgtagtccataaaccataatcccattttaatttaaatacgtcgagtgtcataccacgcacaattttaaccatttttcgaccagtagaaaaacgtgttaattcttgtactgtgcctaatgtttgtgttgtagggtatacattgataaaacaaccagcgtctataatttttttactaccattcattggcatatttttaagtttgctagctgtaccaccgtcaatataataaaatcctggttgtgttaagtcgtttaagtcgtcaatattgtctggaatagataatgcacgtccatcgtcttttgttaatttatagttttgtgaacctctcgcacgtaatgcttcaaagtgttcatactcaccaagttgaaagaacccatataaattattgaatcgttttccaccaccgccattagtcatagcaagtaataacgatttacgttttgtttttggattggtataaatacaaataccctccggctctttaaagttatcacgtggaaaattaataccgtcttgatatgataatttaaacggataatcataaatcttttgaccagtggttaatgaatatttaccaatttgaacgtgtgaattaactgaactgttaccacttaaccagtataaatcatcaccatcaacggcaatcccttgcatccatcgattatcattgttttctgaattatcaatcgtcatttctttttctacattatcaatgtgattttttacgtcagctcttgaacgtacctgtattgtcccgtcaccgaatcttaaaacgattttgtcatttgcttcatcgattaaaggtgtaaacgtatgtttgtttaaaagtgactgtggtgtgtaatctgttaaacctttagcctcttctaaatctaatacataattatctttatatgcgacttgtaacagtttcgcgacaccgtcatgatgtaaccaaattttcatttctccattggattgacgttctaatccgattgttgtaccgtgaccaccttgtacaatacgcatactagaaattaagtcaccgctaggcgttaatttattaatccaaaaaccttctgggttttgtgaatctgattgtgtagagtacatttgattcgtttctttatcgatattaattgattggtttactgcgttacgaataccaccgaagcccataacaaactttggttcaagctcatttaattcaaaaccattaactaaacggtcaatgtctttaattaggtctttcacttctgctttaaaatcattcatttgtttcatttctgcgactttaaataatgcaaatgcagatgttaaaccagcactatatttagtaaactcatcgtgaatgattttatcaatcgtaccgtcgtttaaccaacctctaaataagtcttttgcttggtctgggaatgctttcattaaatcgtcccagtttttgaaacgtttttttaactcaccgtcatagtcccaaatacgatatgctaatacttcaatgagttttgataatcttgaaatataatcataatatgattttgaattggtattataatctgctctatcatcgtaaaacggtgtgtaacgttctctatttttatatatttcgtctaaaaatggacgaatgtcgtcaaaatatttaaattcgttttcattatatgccataattttccacctttaccaaatttgtaaaaaacattttttatcaaattcatttaaaattttctttcttaaatcgtatactttatcaatattatcaattaaatactgttttgaaaattgtgtacctttcgcattacctttttgattttgattacgttttgcgttttgattactttcgttacttgatttattcacagttttaccgttatcaattgtattattgtctgcaaattgtaacgttgttttatcaacatctatgttaacctcgctttgtggtaatgacgcataagcatttctgttcgctgtcataccagttgaattgtctaaagatgtagcattttgatttgaggtttcatctgtgttgtttgttgtatcttcattatgttctgtaaaaccttgtgattgtagatatttttcaacttcgcttgatgaataaaccacattcaaataatcttcatgtgtgatacatacagtaatcacttgcatgccaaacgcttcaactgtttgtctgttgatttctctatctaaaaagtgtattgtaaatgattttttgaaaagtaagtcagataagtcatctttaagtttaaaacctttaaacactttttcattaacgatggctaaaacgtctttgtcaaacttcaacattttttgcatgaattgaaattcatcatcataaaacgttaatttatcattatttacaaattcattaaaaccttttttaattaattctgatttaataaaatcaaataaagtcattgtatatctagccattgtattcactactttcatcattagacaatgtatctatcattgtgatttctgaagtaacttcatcgtcgtaatacggtttaatatctaaaccataacgttttgataagaatgtaatcggttcacgaccttttaaataaatattactatttgatgtggtaaaacctcggttgctttttgcttcttcgtccgaaacaccgctttccttatccactgctagtgaattaatacccaaatagttacttaattcactaattttattttggtattctcttttcatctcagttagtgctggaatcacactattactggttaaatctatgatatcatcatcggcgttaaacataggtgacattttaacaaatggtgcaccgttatatatttccgatacaagttgattaactgactcatcattaatgtctgatttaaatattttgctaaattttgcttgcataattaatgaaaatcgagataaaacaacctcagataattcatcagtataatgttctataatttctatatcactattatattgaattggtttattttgcatgacaacaaagttgccactcatacagttatcatatattttatgaatctgtaagcattcatctggtattaaatagtctggaacaatgaaataaatatcatcttttgttaatcgtttttgaaattgaaaattgaaatttgatgaaaagtttggggcttgattaaaataagtgttgttaacatagcccaaaatcatgatttgttcatttcttgctttaccaacaacaacattaatgttttgccttaatgcagattctaattgaataaaatctataccaaccgaatctcgattggtatagttaattaatagtggtaaaaattccaaataacgattaaacataagacgtttaaatctgttgcgatgttctacaacacgtttattgatttctttagataattcaacctgtacgcctttattatgtttagtcatttatagcacctctataattctgttctcggtgtaacatcttggtcagtaattaaaattttattaaagaatgggctaatggctttaaatgaataataatgaatccagtgtgtgacttcatcaaattcaccattatagaatggttgttttaacataccttttgtgtaacgtttatatttaattgaattaatatccaaaataaatgcgtataaatctgattttggtttaatttcttcaacgttagacttaaattcagataaatttgaaacatcataagtgaatactgaaccaactggaattgtatcacctttatgagtttgataatcaccgtaagcacgtaagaaattaactgattcgtcacttgatacgacaatatctttagtaactttaaaaactccacctaaatcatcaaaactaataacgtggtctgtaaagtcaatccctgctacttggaacgtgttagcaatctttgtatctaaaagataagattttaagctatcagtcgttaaaataacaatatcttttaattttgaaactgttgtatattgtccaatagcaccacctgaagcacgatgaacttcattatatttagcactgttgttttgtaagttaagaatagcttcaaaaactttacttgctaaatcttcttttgatgttgctttacgtacatttgattcagataattgattcaatgaataatcaactaacattgcacgcatttctttttcttctaatacgttaatatcagaaattttctttttatagacacctaatgcataattagttgcgtctgctaatgtttggaaattgaaacgtgtatcattgttatttaatgtaaatttttgtttcttcacaataccactaccatataacttagtagccatacgtgggtagttacgtttcaacattagttcttcatttttagataagtccatgttaataggtactgtatccataattacatattcttcactgtattgaccaataaagtcctgctctttagctaaccaattaaaacggttacctaatgcaatatcgattaataacgtttcattaatcttagggaataaaaatttatttacaaatgtttcaaacattgtattagaattatcccacttatcaccaaacgtccatgattttgaataagtatgattaaagtcttgtaatgcagatttagctgactttgcaactaatagtgctgtttcgttttttgtactcttttctgccatgatttattattcctcctctacatcgccagtaaatgactgttttgaaagtgaatgaatttgtacaccataactatcttcacttttatttgtatcaattgacatattttcatttaattctgttcgtttatttaatcttgaatcttcatatgatgtacccatcatagaacgcatgttgttaccctcgtacatgtttaaattcctcctaatctaaatctaatttatcgacaagttcttcatctgaatagtctttatcattgttatctgtttcatttgattctggttgtggttgtggttgtggttgttgcatttgtgatgtttcaaaattagtaaatcgttgttctaatgaagcgatacgttgttctaaaacaactgggtctaattttgcactatcttcatctgttatagtaggttctaatttgttttcattttcttcttcgattgtttctactgttttatcttcagttgattcttcagttgattcttcagttgattcttcagtttcttctgttgattcttcagttgattcttcagttaattctttgtcgtctgattttacgatttcctcaaattctgtcatttagacacctccaaatattttataactaattatatcatagaatatttaaataagtaaattaaatttattttaatttcaaatcataactttgaataaaagtcaatagatacataaa

SEQ ID NO: 3 - DNA, 42966 bp, Bacteriophage Pseudomonas aeruginosa DSM 34648
  source 1..42966: mol_type = genomic DNA
cgcggggcttgcggtatagtgaagccaacgacgtataaactaggccgacactatgtccgacgaactgaaagaaagcgaagaaaaggccgcatacgcggcccttcttttgaaagaacgcgacccgtttaaggctgcgctttcgctgtttccgaacaacacgaatcgcgcgctatgggttgcgaaccattggccgaacgacgccgaagttaaggccgaacaaaagcgccttaccgacgaaggcggcgatatggcatttcttccgggcaaaggcgaccttgcccgcgacatttggcagcgtatgcaaggtacgacgcttccgaacggcgtaaccattccgccgacgcccgaagaatacgcaaagcttgccaagctttacgccgacgttcgcgggttcatcgaaaaaccgcaaacgaacgttaacgtaacgacgaacgtaaaccgcgtcgtcgaaatgcccgtattcgctaacgaaagcgaatgggaagcggaagccgcacggcaacagcgcgaattgttagaaaatgcacgcactcgccattgatacgaacggggcgaaacctgttccgtatgaagtcgtatttaagccccttccggggtcgcagactatcgccctttgttcgatggcagcgcatacgctgtacgaaggcgcacgcggccccggcaagacgcttacgcagcttatgcgcttttatcgtaacgtcggcaaaggctacggcaagttctggcgcggcgttatcttcgatttggaatttgaccatttgggcggccttgttgccgaatcgaaaaaatggttcggcgataacggaaagctaaaagacggcggcaagttttacgaatcaacgtcggcttataaatgggtttggccgactggtgaagaactgttgtttcggcacgttaagaagctgtcggattacgaaggcttccacggtcacgaatacccgtttatcggttggaacgaacttacgaagcatccaagcggcgacctttacgacaaatttatgtcggtcaaccgctgtacgttcgacccgataaaagacacgccgaaagacccgaaaaccgggcgctatttgacgccgaacggcgaaccgctgccgcctgtaaagtgcgaagtattcagcacaacgaacccaagcggccccggtcacaattgggtaaaacgtcgctttatcacgattgccccgcgcggcaccgtagttcgtcgcgaaattcagatttacaacccggcgaccgaaaaagaagaaacgcacgtaattagccaaatcgctatcttcggttcgtataaggaaaacccataccttccggcttcgtatatcgccgaactggaaagtatcaaagaaccgaacttgcggaaggcttggctttacggcgattgggacgttaccgcaggcggcgcaatcgacgacctttggcaatcgcatatacacgttgtaccgcgcttcgtcattccgccaagctggcgaatcgacagaacatacgacgacgggtcttcgcatccgtttagtgtgggctggtgggcggaagcggacggcaccgaagcgaccatagttctttcggatggcaccgaatttacgttttgcccgcaacccggttcgcttattcagttgttcgaatggtacggatgcgcgaaagacgaaaaaggcgaatacataccgaacaaaggtttgaagctttcggcgtcgaatatcgcacaaggcataatcgaccgcgaaatttcgctaatggcgaacggctggatttattcgcagccttggcccggccctgccgacaatcgaattcgccaagtaatcgacagcgaactagacacgaccgaaaagcttatgtcgaagaagggcgttcgctggactgaatcggacaaatcgccgggttcgcgcgtaatcgggttgcagcttttccgcgaccggctagaagcgtctgttaatcgcgaagggccgggtatatactttatgtcgaattgcgttgcaagtattgatttgctgcccacactgccgcgcgacgaaaagaagattgacgacgtagacacgaccgccgaagaccattgttacgatatggtgcgttatcgcgtattgaaaggcgcgaataaagcggcagcgaaattcaaacttgttatgccaacttaaaggaacccaaatcatgccgaacgtttcatttattcgccccgaacttggtaagctgttgccgctgtattacctgattcgcgacgcaatcgcgggcgaaccaacggtaaaaggcgcgcggacgacttatcttccgatgccgaacgccgaagaccaatcgaaagaaaataaggcgcgttacgaagcgtacttgaagcgggccgttttctataacgtagcccgtcgaaccttgttcggcttggttggtcaagtgttcatgcgcgacccggttgtaaaggtgcccgcgctgttgaacccgcttgtcgcaaacgcgacgggttcgggtatcaaccttacgcagcttgcgaaaaaggccgtatcgctgaaccttgcgtattcccgcgccgggctgttggtcgattacccgacaaccgaagccgaaggcggcgcgtcgattgccgaccttgaagccgggcgcattcgtccgaccctgtacgtatattcgccgactgaaattatcaattggcgaacgaccgaccggggcgcggaagaagttttatcgttggtcgtactgttcgaaacttggtgcgctgccgatgatggctttgaaatgaaaacgtcggggcaattccgcgttttgcgtttggacgaagaaggttattacgtccacgaaatttggcgcgaaccgcagccgaccaaagccgacgggtcgaagattccgaaaggcaattaccaacaatacacggtttataagccgacggacgcaaacggcaatcgtcttaccgaaattccgtttatgttcatcggttcggaaaacaacgattcgaacccggacaacccgaacttttacgaccttgcgtcgctgaatatggcgcattaccgcaattcggcggattacgaagaaagttgttatatcgtcggacagccgacgccggttcttatcggacttaccgaagaatgggttacgaacgttcttaaaggttcggttaacttcggttcgcgcggcggtattccgcttcctgccggggccgatgcgaagttgcttcaagcatccgaaaacaccatgcttaaagaagcaatggataccaaagaacgccaaatggtcgcacttggcgcaaagcttgtcgaacaaaaggaagtacagcgcacggcaaccgaagccgaattggaagccgcttcggaaggttcgacgctttccagtgcaaccaagaacgtttcggcggccttcgaatgggcgttgaaatgggcggcccgttgggtcggccaagccgacagcggcgttaagttcgaactgaatacagatttcgacattgcccgcatgacgccggaagaacgccgttcgcttgttgaagaatggcagaaaggcgcaattaccttcgaagaaatgcgaaccggcttgcgtaaagctggcgtcgcaaccgaagacgacagcaaggcgaaagaaaaaatcgccaaggataccgccgaagcaatggcccttgctgccccggctaacgtgccgggcgatggcagcggcggcgataatgtgggcaacaacggataaggggcgcaatcatggcactatcggacaataagcgtttgtacgatattgcgacgcgccttgctgtttacgtcgaagacgtgaaagtttggcagtcccgacaattcgggttcgtacttcgcgaagtaaacttggaattaacgcgccttcttggtcgtgttcgttataagacccttgacggtctttcgaaggcgcagttaaacaagcttgtttcggaattacgggaatcgcaatcgaagatttacagcgcatacacgcaaacgctacttgaacagttaaaggaattcatgcgggccgacttggaagtaaaccggcgcgcatgggttacgggttatatcgaacttgacggcgaagaaagcgacggcattatttcggacgaagaagcgatacagtttcttttagaagtacccaacgccgattcgaaccctttgttcggtttggccgctgttacaggaagcgacgaacgcatttggtcgcaagttacgaatacgccaattcctgcaaatggtttgtacttgctgccgtttatcaagacgtttacgaattcggcacaagctggcgtcgaaagcatgattcgcaaagcttgggcgaaccgttggacggttgaagaaaccttaacggcgcttgtcggcgatggaaccgcagcgcagggcacgccgtcgcagttgcaccgggtcaacgcgcaagccgcgtcggtaatccatacggcaaccgcgcacgttgcggcggtcgttgcggctggcgttatgtctgcggttttcggtcgttacgtttggtattcggtaatcgacggaaagacaacggacatttgcataagtcgaaaccgccgaatttatcgcttcggcgaagggccgttgccgcccgcgcatatccgttgccggtcgcacgttgccccggcaaataccgctagtgacttggccgaagaaacgttttatacttgggttgcccgtcaacctgcccaagtgcaagacgacatattaggcgacgaaggcggcgaagctttgcgcgatggtcgcttaaaggcgaaggatattccgaagtatgatgcggacaggccgctaacttacgaagaattccgacgcaagattaaagaaattctttcccgctgattcggtgaatcggcataaccgcaaggagtccttgaaatggcactgaaaaagaaacttaccaaagaagaacacgctaagctttcggacgcactgaaagccgaatatatcgaagacggcgacggcttccgccttgacgttgacggcgacgaagatacgggcgctttgaagcgcgccaaagaccgcgaagcgcagttgcgcaaagacgccgaaaaggaagcgaaggaacttcgcgaacggctggaatccatcgaaggcgacgacgcgcgcaagaaaggtgacattgcgacgcttgaaaagtcttggcaatcgaagcttgaaaaacagcgcgaagaatacgaagccaaggtttccaagcttaccgcgcatacgacgaaaacgcttgtcgataacgtcgcgtcgcagcttgcccacaagatttcgaacgccccggcaatcatcatgccgcatatcaagtcgcggcttatcgcagacttcgaaggcgacacgccggttacgcgcgttctggacaaggacggcaagccgtcggcccttactatcgacgaactggcaaacgaattcgttgcaaacaaggatttttctgctattatcacggctagtaaggcgtccggcggtgccggtaagccttcgcagaacggcggcggtgccccgaaatttaacggtcaatccgacaaacccgccgacctttcgaagatgaatcccgcagaacttgcggccttcattaaagaagcgaaggcaaccgaaactaaggacgcttaatcatggcactttccgaccttgctgtttactccgaatacgcttattcggctttctccgaaaccctgcgccaacaggttgatttgttcaacgctgcgacgggcggggctatcatgctgcaatccgcagcgcaccaaggcgacttttccgacgttgcctttttcgccaaggtaacgggcggccttgttcgccgtcgtaacgcctacggttccggcaccgtcgccgaaaaggtcttgaaacaccttgtcgatacgtcggttaaggtcgcagccggtacgccacctgttcgccttgaccccggccaattccgttggattcagcagaacccggaagtcgcaggcgcggcaatggggcagcaactcgccgtcgatacgatggcggatatgctgaacgttggtcttggttcggtctattcggcgctgtcgcaggttcccgacgttgtttacgacgcgaccgcgaacaccgatgccgccgacaagctgccgacttggaacaaccttaacaacggccaagccaagttcggcgaccaatcgtcgcagattgccgcatggattatgcacagtacgcccatgcacaagctgtacggttcgaacttgaccaacggcgaacgcctgtttacttacggcaccgtgaacgttgttcgcgacccgttcggcaagcttcttgttatgaccgattcgccgaacctgtttgccgcaggtacgccgaacgtttatcacattcttggccttgtgccgggcggcgtgttgattggtcaaaacaacgacttcgacgcaaacgaagaaaccaagaacggcgacgaaaacattattcggacttaccaagccgaatggtcgtacaacatcggcgttaagggcttcgcttgggacaaggcaaacggcggcaagtcgccgaccgatgcggcgttgttcacttcgaccaactgggatcgttacgcaacttcgcataaagaccttgcgggcgttgtcgtcaagaccaactaaccgacggcagacggacggggcttcggccccgttcttctagtccttcacaaattcaaaggagtttcgaagatgaaaccggcaaaaattctgttcttcgttgacggcaacgcaccgaccccggaagacttcgcagccgccgccgaactgaacgcgcaagttatgttcaggaacgcccgcgctgttccgtccgaaccgcattcgctggaaatctgcgacggcgtagcgggcaaggttccgaagctgtacgccgacgcttacccggaagcgggcgaagcaatcaagaagaaggccgccgaactgaaagcccttgcttcgaaggtcggcgacgccccggcaccgaaggcggccagcaagcccgccgcagcgcccgccaagggccagaccccggcgcagggccagcaagccccggcagcggccccgcagggcggcagcgccccggcttggaaccccaacccggcgcagtaaccaacggacggcctgtcgcttattgtgggcaggccgtttcaacaacgaactaaggagtcttcgcaatggcaacgaaaaaggttgtttatttcacggcaggcattaacgcaacggctggcgaacttgccgacattgcgaagcttaacgcagccgccgaaccgcaatacgaagttttggtagccaacggcgcagcaaatgccgaatacggcgaaaccgaccgaattattccggctgattttgtcgcgggtacgattcccgacgtttaccgcgttgacggcgacccgctggaagacccggtttatcccgaaatcgaccccgacgcaatcccgaatcaggcgcttacagcaacgcaggcaatcgttaacgacgcgcaagttctggacgttgacggcggcggtactgttacgcttaccatcgaaggcggcgttattactggcgttgtttacgccgctggcgaataaggcggttgacgcatggcaattacaatcgttgttgaagacggaagcggcgtaacaaacgcgaacagttacgtaagcgttgcagacgcgcgcatttacgcttcgaatcgcggcgtcgaacttccgttggacgacgacgaattggcggccatgctgattcgttcgacggattacctagaagcgcaggcttgccggttccaaggcaagccgacttcgacaacgcaggctttgcaatggccgcgaactggcgtctttcttaacgaagacgaagtaccgtcgaacgttattccgaagtcgcttattgccgcgcaagttcagcttgcaatggcgattaacgcaggcttcgaccttcaaccgaacgtttcgccgcaagactacgttacgcgcgaaaaggtcgggccgattgaaacggaatacgccgacccgctgtcggttggcatcatgcccacatttaccgcagcgaacgcacttcttgcgccgctgtttggcgaatgcgcttcgaacaagtttgcgcttcgtacaataagggtttgacgaatggcacgtttcgacgcagcaattaaaacggcgcaacgccttatcgcaaagaacggcgaaaaggtgaaatggcgcgttatcgaagacgcgacgccaacagacccgaacaagccttgggaacccggcccggcattgccggacgacaaagacgttaccatttgctttttgccggttgaccggcagacgcaagaaaccttcaacttcattaaaggcaccgaagttccgaaaggttcggtaatggggcttatgggcaatgttccgtttgaaccgaatttgaaagacgttgtaattcgtaacggggtcgaacttcgcttggcttatatcgacgtactttcgcccaacgggcaaaaggtactttacacgatggtatttcaagcatgattgaattcgaccaagttaacgacgaagtaaacgcgctttttcttgcagcttggaacgcaggaagcgcggcaattgcgggttatgttcccgaaattcgttggcagggcgtgcaatatcgcgacttgccggacggttcgaagttttgggttcgactgtcgaagcaaaccgtttttgaagaacaagcgaccctttcaacctgcgaaggagtaccgggaaaaagaaaatacacggcgtcgggtcttgtcttcgtacaaatcttttgcccgaaatcgaatacgcaagcgttcgaacttgggcagaaattggcgaagcttgcccgtaatgcttttcgcgggaaatcgacgccgggtaaggtttggtttcgcaatgtgcgaattaacgaacttccgcccgaagaactttacgaacggtttaacgtcgttaccgaatttgaatacgacgaaataggttaaggagttcttaacatggtatgcgaaattgccaaaatcgacagcaacattaccggacttgccttcgccgaagaagaatgcttgaagcaacttccgacgacgcccgtttggtacggacttgaacccaacagctattcggacttcggcggcgaactttcgaccgttgcccgcgcgcctatcgacccgtcgcgccagaacaagaaaggcacgattaccgaccttgacgcatcgggcggcttcaacgccgactttacgaagaccaaccttacgcgaattctgcaaggcttcttctttgcagacgcgcgcgaacttccttcgacgcagccgcttaacggcgcatcggtcgcgcttaccggcgttaccgcagccgacgacacttacgccgcagcttccgggcttggcgtgttcggtgccgatatgttggtatatgcgaccggctttgccaacgcggcgaacaacggccttaaaaccgtcgtttcggctaccgctgcgggcgtcgttgttgccgaaaccttgattgacgaaaccccgcccgcaggcgcgaagctggaatgcgtcggtcggcagcttggcgcggcagacgcgaacattgccgtaactggcaacgtcgtttcgcttatcgtcaccgctggcgactttacgaccatgcccgaactgttccccggtcgttgggtcttcgtcggcggcgatgcggcggcaaaccgcttcgctaataatgtgggctatgcccgcattaagtcggttgcagcgaaggcgcttgttttcgacgacgtgacttggcaggctgccaacgaaaccggaaccggcaagtcgattcgtcttttcgtcggaactgttatcaagaacgaaaagaccccggcatttatcaagcgtcgttcgtatcaaatcgaacgcaccttgggcgaaggtttgaacggtacgcagtgcgaatatctggaaggcgcagtaccgaacgaatttacgttgaacattccgcaggccgacaagctgaacgccgacctttcgtttgttgcgtgcgacaacacttaccgcagcggcgaccccggcgacgaacagaaagccggaacccgcgtgcctgcgcccggcgaagatgcttacaacacttcttcggacgtttaccgaatcaagatggccgttcacgacgccgcgtcgtcgaaccccgccgccctgttcggctacgtttccgaagcgaacgtttcgattaacaacaacgttacgccgaacaaggcggtcggcgtgttgggcgcgttcgatacttcggcgggtaacttcgaagtcggcggttcgattaccgcttactttacgaccgtcgcagcggttaaggctgttcgcgcgaacgccgacgttggtttgtcggtaatcagtgcggccaagaacgccggtttcgtgttcgatattccgttgcttggtttgggcggcggtcgtctgaacgtcgaaaaagacgcgccgattaccgttccgcttgaacccgcaggcgcagaaaacgcgaacggttatacgatgttgtacgaagtgttttcttacctgccgaatctggcaatgccggattaattgcggtaaacttgaagggccgggtaattccggccctttcttcattcaatcggagtaaatcaaatgtctggactttttaagcaattcaaaacgaattcgaccaaggaagccgaaggcgtcgaaatcgaatttcccgaagcgcagaacgacgacggcagcgttccgactttcgttatttcccgcatgggcaaatcgaacaaggcgtattcaaaggcacttgacgcggcgacccgtccttatcgccgtcaagtcgaacttggcacgctgaaaaacgaagtcgccgaatcgctgtttatgggcgtgttcgtcgataccgtgttgcgcggctggaagaacgttcagggcgaagacggcaaggaaattgcgtattcgaaggacgccgcaatttcgcttctttccgaactgccggacgtttacgaacgtttgcaggaagaagccaagttggcttcgaacttccgcgataacgctttggaagccgaagcaaaaaactaaccgaagttttggcgcacctgttggaacttggcccacacgaacaggcgatagcaaagcaagcgatgcgcgcggggcaaccgttacccgaacgcatcgcgaacgcgccagaacttgaagtaggcttgcagttgtatttgcaagccttcttcgacctagatagcgaacggtcgcacggcaacggtttaacgccgataccttggacaagtatggcggcttacgcaagggctttcgagtttgacgaagaacaaaccgaagacttgttttattttatgcgaaagcttgattcggaacacttgaagaaactagcggacaaacagaaagcggcggcatcgaatggcaaaaagcctgctagacctagccgataggctggaaaagaaagcgaaggcaatagacgaagcggcgtcacaaaacgccgtcgataccgctttggctattgtgggcgacttggcgtacaaaacgcccgtagatacttcgcaagctttgtcgaactggattgtaacgctagaaagtccgtcgggtcaacaaatcaagccgcattttccgggttcgcagggttcaacacaacgcgcttcggcggctgaaacgttgaattctgcgaagcttgttttacgaaataagaagcccggccaagcgatatttattacgaacaaccttccgtatatccgcaggctgaacgacggttattcggcacaagccccggcggggttcgtcgaacgcgccgttttgattggtcgcaaaatgcgtaagaagttcaagattaaggattagaagaaatggccgacgaaaacatagaaattaaggttcaagacaaagtttcgccgtccatttcgacgaagcttcgcacaattgccagcgaagcccgcaacgccgacgccgcagttaagaaccttcaaacgcagctttcggcaatcaacgtcggcggcttgtcgcagcttatcaacgcatcggccagcgcaacgcgccagcttcaacaaggcgcgcttgccgcgcaacggctggcaaccgaacagcagcgtaccgcaacagccgcagcgcaggccgccgcagcccaacagcgcgtcgcgacggctgcaacccaaggggcaaccgcgcaagccaaccttgccagcgccacgcagcgcacgcagacggcccaacagcagacggcgacagccgcgcagcgcctagcgacagaacagcagcggacagccgttcagacggccaacgcggcggcagcgaacgaccgggccgcccttgccgccctgcggctgcaacaggcgcaagaccgggccgccaattcgacccgcaacgcgacttcggcccttggcggatacattcgaaccgctgccggaattcttggcgtaacgatttcggcgaacgcaattcttgcaagtgccgacgcatacgttacgcttcaaaacaagttgcagaacgtaacgaagtcgcaagaacaagttaacacgcttacgaacgaacttttcgaactgtcgaaccgcacgcgcgcaggcattgaagaaacggcgacagcgtttacacgcttcgaccgtgccttggcgtttatgggcaagtcgcaagaagattcgctgcgaatgaccgaaaccattaacaaggctttgattgtttcgggcgcaacagcgcaagaagcgtcgtcggctttgttgcagctttcgcagggtttcaacgccggtaagttgcagggcgacgaattccgcgccgtttcggaaaatatgccaatcgttttggacgcagtagcgaaggcgcttaacgttccaatcaaccgcgttaaagaactttcgaccgaaggtaagattacttccgaagttctgtttgaagctttcaagcttatacaagaccaagtagacgcaacgtttaacaagacgacgcccacaatcggccaaagcttgacggttcttcgcaacaatgcaattcaattcttcggcgaattgaacaaagcgaccggatttactgccgggctttcgcgcgcgattctttggcttggcgaaaacttgaagacggttgccgtaatcgtcgcagggcttggcgttgcgttgcttgttgccttcggtgccccgttgaccggtgcgctggccggtgcgacggctgcggtaaaagcctttacgctggcgcttgcttcgaacccgattggccttatcgtcgtcgcgctttcgactgcaattgcgtatctaacgcttttccgcgacgaaattaacttgggaatcgacgacgttacgacgttgggcgatttcttccgcgcgacctttgaaggcatcggccaagcaatcgacgacgttaaaaccatcgcgtcgcaattgtgggcagaacttagcgacttcgcaagcgcagcccttggcgaaattacttcgaacgttgacgattcgacttcttcttggtcggacagctacgccgcattctttcaaaccaaccgtacaggttgggccggtgcgctggaaaacgccgcaaaagttcttgacgcaatcgccgggcttttgaccggggccgcaacgttcgcaggccgtgcaatggccgaagttgttatttcggttcaaaacggaatcgcaaacgcttacaacgttgtcgcgggttggattgaaaacgtaacgaataaagctattgaagccgcgaacaggcttcgcgcgatggtcggtaagtcggcttatgaacttgtccaattcgaacgcatgggcagcgcaggccaaaccgaattcgaatcttggggcaagctttgggcgcaatcgctggaagacggatttaacagccaaggcggcgcaatgcaaaacctgttgaacggccttttcgaccgttcgcagcaaatcggcgcgcagcgcagggccgcaggaagcgcgcagcttcgcggggccggtacgtcgcagcttgccggggctaccgacgcgaacgcggcgaaggctgcggaacgtcgcgcgctggcaatggaaaaaatcaatacgcagcttgacaacgaattggcgcgtatgttccagcttcaaccgcagcgcgaagcgcaagcgaagttcgaccaaatcgaagaaagcttaattcagaaaaagattaagcttacgtcggaagaagccgaagcaatcaaggcgaagattaaggccgttcaagatgcgaccgaagttcaacgccagttcgacgcaatttacgccgaagctgttaacccgttgaaggaatacaacgcggcgcaggaagcggcgaacaagcttcttcaaatgggcgcaattacgcaggaacagcacgcccgcgcagtaacgaaggcgtcggaagcttacgcaaattcgcaagacccgttgcggcagtataaccgcgaccttgaacagcaattgcagcttttgcaaatgctgccgaagcaacgcgaaatcgaacagcaagttatgcaagttcaaaacgacttgcttgcaaagggcatcgttctaaacgaaaccgaattggcgcagcttcgcgaaaagctgttgcttattcagcaagtaaacgccgtttcgcagcaagaagcgtcgttgttagacgccagcgtaaacaagcgccaacagtttatcgaccaacttaaagcaattcagaacttgcgcaacaacagcggaagcggtttcaacgcaggcgaccaagccgaagcaactaacagcatgttgcaaggtatgggcattgatacgacgaactttcaaacgcagcttaacgcgcaattggcgcaatatcaaacttacgtcgaacagcttaaaatgctgaacgaacagcgtttgattagcgaccaagaatacgccgccgcaagtatgcaacttgaattgcagcggcaaaacctgtacttgaattcggcaagtagtttcttcggaaacttggccgcgcttcaacagtcgggaaataagaaaatggcggcggtcggaaaggccgcagcaatcgcgcaagcgatgattaatacgtatcaatcggcaacgtcggcttatgccgcgatggcgtcgattccttacgtcggcccggcgttgggcgcggctgcggctgcggctgcaattgccgcaggcttggcgaacgttcagcaaatccggtcgcagaataccgggtttaagtcgggcggctttaccgggtcaatgggcgtaaacgaagtcgcgggcgtcgtacacggccaagaattcgttatgaacgcatcggcgaccaaccgcattggcgttgcagaccttcaagccctgcaaacgggcgcggccagtgttcagcgcaacgacgaacaggcaatagcggctagtgtgggcaggggcggcaattccgaaccagcgcccgcgccggttgtcaatgtaccttttagcgccgttgtcgtacaatcgaaagaagcggccttggccgggcttaaatctgcggaaggccgggctttcattctggaaactatcgaacaaaacggcggcaccgtcgcaaaaatcgtcggagttaaataaatgggttatgcaattggaacagttacaaaaagcggcggcgatgattgccataatcaaatgcttggcgttatcaaaacgttggccgaagctaacggatggacgacgcttcgttatatcaacagcggttctaattgggaattgatactaaaaggcgtcggcctttctggaaccgaagaaatttttgtagggtttcgctgttatcaaagtacaaccggcgactattataacattgattgcggaacctttatcggatatatcgcgggcaacgcatttgcggcgcaaccgggcgcgtacatatattcggtgcctgccaacaataacgcaattacgtattttataacggctaacgcgcaaagaattgtcggatgcttcaaagtcggcacgccggtttatatgcacttctacgtcggcaagttctttccgtatgcgcgccccggtgaatatccgtcgccgcttgtttgcgcggcaatgctaaacgcatcggacgcaacacgtttcgacaacgtgaatattacttttccgtatccgggctatcgctaccaaacaacttgggtaaagcttcgcaatcgcgaccaaggcggcaactggattcagccgaactgttatccgttcctgcaaaacagttcagcgacgaacgcgcttgcaggcgtgcaaggaacttcgaccttggttcctgccgctactttctaccaacttgaaccaataatattgcagcaagacaaaagcgatattgaaccaagcaacgtttggggcgaattcgacggcgtttatttctgttccggctttaacaacggcgtcgaaaacgtagttcaggaaggcggaagttctgtcgttgaccaaaccgggcttaccgtacttcaagccgtagacgcaattaaagcggtcggcgggcgggcgtttgtaatgttgcaaaacgtctatcgtacttcttggcgcgattttatcgctttggaaatgaaataatggcatactttacaggaacagccgccacaatggcggacttgaaaaccgcaattgaaaacgcagccgtcgccgcaggttggacgctaacaagcggcattctgtcgaaaggcggttgcttttttcaacttgtcgcaaaccaagtaacgaacccgtatcttcgtcttttgggcggaaccggccaaagcggttcgacgcttaccggccaaccggcgcaaggcgtacaaatcgcaagcgcagccgcgcaagttatggtttttccaataaattacgaaatatacacgttttccaacccggacgaaatttattgcgtagttaattataattcggacttttaccaacaactttcgttcggtaagtcggatattccgggcattggtggaactggcgcatggttgaccggaacttatagttcaactgccagccttaccaacgcgacaagttcggcgcaaatgtatttaagcgtaaaccaaacgtcttggggaaacacaagcggaaaccaagtaatcggcggctttttcttgggcggcagtacgggcggttgttcaagcctatttcattgcggtttggattccgtcgcatggcgtcttgacaattcaagaacagccggaagcggcgtacttggctgcgattactgcgcttcgttgattaccgcacttccgaacgtttcgaaccaagcaacaattttgcttccaattaaaggcatggcggttcgctttgacggcgggcgaacaattgtcgtaaatccgaaaaatgcgcgttatatgcgaaacgataacgttgttccgggcgaaattattacgttcggtgccgaccaatggaaatgttacccgttcttccgcaaagacgcgaccgttcgaaatggcgtttcttggtcaactggcgcgcaacatagcggaactttcggctatgcaatccgatacaatggaagctaacaaatggccgcacgttctggaactttcgcaggttcgttcagtttcgaatatggttcgcaaaatccgaatatttcggaagaagtggccgaatatagcccggcgcaatatgcgccgcttgccacgtatgacccggacaaaccgcgttcggtagccaaccgcactttttacagaatagcgccttcgaatcgctggcctattgtgggcaaagaacaaaccaacttcgggcgcgattattattatcgtgttcacgtttcgccgttgttcttggacttgcaaacggtcgcgtcgtcgcaaacgcgcgaattcaacgtttggaacgcatggcccgaccgtgcggcgaatcttgacgacattttggtaagtaatccggtcggtattgaaattacaggccaagcgacgccgtatgcaatgccgccgcttcaagaacttacttacgaaataacagtagggacaagcggcccgccaaatattaacgtcgaagttcaatttgacttttccaacgttcccgacccgctgccgattcttattacaggaacgcgcgcggtcaagttcgacattgtgcccgaagttccattaaacgaaacttgggaatggttaagcgacaacattgtagcggttgacggaacagaacagcgcatagcacttcgcggcgaaatgccgcgtattgaagaacggttgaaagtaattttcgattctgtcgaagccgtgcgccgtttttacggcgacgttatgtcggcagtcggtcggctttggattcccgaatttcagtacgcgacccgaattactgtcgcaagcaacgccggtgcgcttcaaatttatttcgaccgaaccaagaccgacgttcgcgatactgaatacgttttgattcaaacgccgcttgttgccgcgcttgtcgaaattgacgtattgacagccgacggggctatgcttggttcgccgctgctgttcgacattccggcagggtcgctaatcattccgggttcgcctgcgcttattgacgacaatacagcacttgcgcggtattccgtcgatactgtcggcgaagtagaaattaacgcgaagatgattcgccagcgttcgcaacttacccgacccggcgcaaccgtcgtacttgaacagttcggcggcgtgccagttttgacgaagcgtccgcttgcaaacgaccttgtacgcgacgaagtttcaaccggccaaatttcaatcgacaatcaaaccggacttgtcgacattattagccgttgggattatagccgcatcggcgggccgcgaagcttcaaagtaaaccgtatttcgaatcccgaagaattggattattggaaagcaattcttgcgtatgcacgcggacaggcgcgcaagttttggatgcccacatatcgaaccgatttggctttggccgtgcaaccgtccgacgcgacttcaagctataccgtcgaagggtcggagtatgccgaaaagatttggccgattatcacgcatcgttatatcgaaatcgaaacagcgtccggcattcatcgaaccgaaatattgggcgcaactttgcttgaaactggcaatacaattcttcttcttggcacgccgcttccgaccggggccggatggatggaagttaagcgaatttcgtacttgttgcctgtacgccttggcgacgataaagtagaatggaagcattacggccttgaatcaatcttgaatctttcaattcgaacggcggaaccctaatgtctgattacgacgacaaagaagaaagcgtaggcgatagcgcgccatttgaactttacgaattcgtcggttcatatcgcaattattatatgacttccgacgttctgtcgcacgtcttcaacagtgcgacatataaccccgttccgggtttgaaacgcagtacgttaaaagtcggaacgcacgaagacgataacgtagatatgacggttacgcttccgattacggaacaaatcgttaaagactatgcgtttcaaactacgccgccgtctttggttttgacgatttaccgtcgccagcgcgacgccgcaacttgggttgcgtactggaaagggccgattgcttcaatttcggttgacgacgaatttgtaacgttcagaacgccaagcaagttcggttcgatgctatcgggcaatataccgaacgtttacgtacaaccgccttgcaataacgttttgttcgacgaacgttgcaaggtaagccgcgtaagcaattcgctagatacgcaggtttcggcggtcgaaggtcgcaacatttcgattccgtcgcttggcggttttcccgacggttggtttatcggcggcgaaatcgcaatacctgcgcgcaacgaacgtcgaatgattgtcgcgcaagccggggcaattctaacggtaaattacgaattcgcgcgtatttctgtcggcacttcggttcaggttacggcaggttgcgaccattcttacaacggggccaacggttgccccaagttcaacaatcaaccgaacttcggcggttgcccgtttgttccgggcgaatcgaataacgtatttcaaagcggggttcattaacaaatgtggattgcaattgtcttcgtcgtcgccttcttgcttatggcggcgcttatgccgaaaccgaacgtcgaaaacgcacgcgcggcgaaacttggcgacttccaatttccgcgttctaagtacggcgacccaatgccgctagtgtggggaacagtgcgccagaaatcgccgataacggcttggtttggcgacttccgcccggtgccaattcgcaagaaaatgaagaccgggctttttagttcgaagaaagttacggtcggttataaaaactatcttggcattgattgcattttgtgccttggccccggcgttcgacttcgcaagttttgggccggtacttatcttgtttgggaaggcaacttaacttcgtccggcgatatttacattaacaagccgaacttgtttggcggcgaagacgaacgcggcggcctgcaaggtacgatttcgttttacgacggtcgttttaacccgccgcaagattcttacttggtttcgaagattggcccgaatgttccggcttacaacggctttgcgcgtgcgttgttcaaagccttttatattggaacaggtacgacgccggaaccgttcagcttcgaaattcagcgcattacgtccggcttgcacgcgacttattcgattatgccaaacgggttggacgttaacccgatggaaattgtttacgacgcaatgacgcaaaaatggggccgcttcggcaaccttgaaagcgaaattgatatgccttcgtttacggcctgcgcgcaaacgctgtataacgaaggcttgggtatgtcgcttattgttcaatctgcgattactggaaaggacttgttagaagaagtaatgcgcgtcgccgacggcgtgttgtaccaagacccggcaacggcgaagattgttgcgaaacttgttcgccaagattacacgatttccgaacttcttgttcttgacgaatcttccgttaaggaacttcgcaatttccagaaaacaacatgggaaaacacttttaaccaatgccgggttacgttcaaaaaccgcgccagtagttacgacgacagcgtagcgattacccaagacttcgcaaatatcaactttcaaaaccgcgttaagtctacggaagtttcgacgcccggcgttacagacgcgacagtagcaagcaagattgcggcgcggcaactttcgattttgaacgttccgctttacaaatgcgatttgaccgtaaaccgcaaggcgcagaacttgcggcccggaagcgtgttcgttctgaattggtcgccgttcggcatttcgaatatggttatgcgcgttacgaaaattgatttcggcgaacttacgtctaaccaaatcaaactttcttgcgtacaagaccgcttttcgtcgtcggcgcttacgttcgcaccgcccgaaggttcaggatggacgccaattagtacggaaccgacgccggttacaacgcggcttctttttacgccacctgcgttccttaccggatacgacgacagcgaaaccccggcttcgttcgattctgccgggcgtctgtaccttgccgcagttgcgccgggttctacgtcaatttcttacgacgcaatgacggccccggacaatttcagttcgtcgcctattctgtcgcttgaaagcgccccgtacaacggcggcggcgtgttgctgaacgcctacgcttcgacagtcgccagcgaaacccgcaacgatacaagcggaagccttgtcgtaaccggcgtgtcgcaagcaagcatcgaaggtttgcagcaatacacgacgctagaccaagcgcgcgacggttcggccttcctgctgattaataacgaactgtttgtttatgtgggcttcgttgacaacggcggcggtcaaattactttcccgaacgtgtatcgcggcgttcttgatacaacgccgggcaatcatgctgcgaacgaccgcgtttggttcattagcggaaccgacggactgttgccggaacttgtttcggtcggaactacgcgatacgttaagcttttggatacgacttcgggcggcaagcttgatatttcgttggccccgtctttcagcgggtcgcttaccaaccgggccgggttgccgctgccgccgcagtacctaacgcttgcaggaagccgcacgccaagcccacaagtaggcgcaacgtcgattgctgttgcatggcgcaaccgcagccgggccgataccctgttgcgcgtgtatagcgacacggcgaacacgcgggaagctggcaccgaaacccgcgttcgctggcgcgtaggcggcggcagttacacgaccgttacgacttcgggaagttcaacgacccttgacgtaacgggcaagtacggcacgctagaagttattgtagattcgtttattacagcgaattcgaaatattcgacgtacagcgattcgcttacaatgaccctaacggcaccgccgccgccgtaatcaaaagaacgacagcgcggcggttttggctttcttcaaccgcccgcagtcgtacagcatttcgaccgcttcgttaatgtaccaatcgtaatttatatcgtcgggaaattccgtcggcaagtccattacagggcgcgcgccgtcggttttcccgactttgtttccgctggatacgtaagcaatatacccggcttcgttcttcgggtaataccaacgaacgaccttgccaagataacgaccgttcttttcgccgccgccgcgcacgttctttactgcaacgaagcgccggaagtcgcggcattccttaattgtcttttcgaccggcgttccgtcaacaaggaaccgaacaacggcgtcggaacaaatcagggtttcggggttcttcgaaagaatcgaattcaaggccgacccgcgttcgcaataagcgcccttcgtttttgcgcccaattgttcgtcaataaagcgcgcttcggggtcgccgccgtcttccttgattgcgacataactattaacgtcgcggctgaatacggctttataccgcgtttcttcggtcttgtatcctgtccattcttcccaagccgcaataagcgcccttacttcgtcgtgtcgcgacttgtgatacttcgaaataatgccgtcggtattgccggaaataacttcaatgccgatttgttccaaagcttcgataagcataagcaacacaagttgcccggtaatcgttacttgcaacataagttgcggcgcgtaaagcgtcgaatacttgttaccaagcttaccgaagcttccgttaatggtaatcttcaaactgtcggcaacggtcttccatttcttcgcggctgcgcggtcgcccgccttctttgccttggccgcttcggctttggcatgaattcgcgtatttacgattttttcgtaaacggttaagaaagcttcgcccaagtgcggcgggcaaagtctttgattaaggattgttcgcgggtaaaacgattctacgtcgttgtctgccaaaattatttcgtcggtcgcatagtgcgccgttttcttttcggtagaatgcaaaccgcccatgcctagtttatacgtcgaaccgccgatggttactttcagcttttccagttcgggcggcatgattggcgaccccaagccgtcaagatagaagcgggcgtttcgcacgacttccagcatttcgcgaagctgcgtcgtttgatagcaaacgaagtcgggcacttcgtaaaccaagaccgtatcggcggatagtgtgggcttcttcggataatagccaaggactttttgaagttcggagttaataaccgcttcggctacttgtgcgtctgatttcgaccgaaggtctacgccgtattcttccgacatttcggcccgcaatttcaattcgggcgcaagttcgttaaacaaaagttcggtattcgaaaggtcgttgcagcaatagggccgcactacttcggcgtcttcctgcgttaatacatggtcttcgggaaatggcaagtcttgcatacgttcgcaatgcaagcgccccgcgtacagcttcaacgaaccttgaagcggcgcaacttcgataaggtcgatatgattgtatcggccaatttgtacgccgtacttcttttcaaacgcgaacggcgttaccttttcggttccatagttcggcccgcttttaatgatgaaatcggacgcttctttaagcttcttgcaatctgcgccgcgtgcggctagttcaatcatcggcaagtcataattgcgcgaattgaagccgacgatacagaaccgccaaagcatccaaagaagcttcgttgggttaaaatcatggtcggggctgcgttcgaacgcgacgaactttccgttatcaagcgacttaaacgccacgtaaaagaaatttacgtaagtttcaacgtcgaagacgaagacacttccggcaggcattgccgttagttcttcgtccgacataaattcgacaggccgcaaagcctgtcgaatgcttgcggccagcttatcgacgacgcggcttttctttgcgacgataaagccttgttcgttaatcatgcgaaagccccttaaaacggtatgtcgtcttcgtaattgtccgacggattatgcgtcgcttcgctgccaaggtcaagacccataagaacgccgcgcaggttttcgccgaaaaatacgaccttgtttgcgtccggtgcgaaatgcgctttcttaaacgcatgttcgacggaaagaagcaacttcgcagaaaagcccattcgttccggcaagccttcgattttgtacgtcgaagcttcttctttgtgcatcttcgacaaaaccgcgccgtcgtcgaagaatacgtttccgttcgggctgaatgactgaatcgcgcgaacgccgttgtaaaaatcgtcgggaaccggccaagggttcaaaccgtcaacttcgaaaacgacttggtaattcgggtaacgttcgccgtaaagctgcgttttgataaacgccccgttttcgaaatagaacgttgccgacgacgccgaaaagccgaagccggtaagggccgggccagccttggcgacagcgaccgccgcgcacttcggaagcatcatgccgggcggaaggtcgataccgtgccacgcttccagcaaggccgccccgttggtcgcgacggcgcttccggcttgcagcaagacggcggcataggtcgcatttggtgcgccgtctgtcgcaagccctgcgaccgcagcgaaggccgttttaatccggtcgtcgattgtggcgcattgcgggtcgggcgcggtaatcggcacgtcgtcgaagcccacacaaggcaccaacgcccggaacgcgccagacgatacggcaagggcgttcgcggtaagctgcgtaatcgacagttcttcgccgaccttcgacagcgcgtcgataaactgcaacgtatgcgggcacgctaccaagtcttcttcgataggatgcgcgacggtcaaaaccccgtcggaagccgccgcccaattgtgggcaatatggccgaactgaacgttcgtcggccccgcttttttctgcgcgatggcaacgaacttcaacgccgccaaaagcgacgccgcagggtttggccctttggctttgttctttccggctgcggcttgcctgcgcgcccttggctttttcttcggctgttcggcggctggcgcttcgtcttcgggcggaagcggaatattactgtcgattttcattttcggccccttcttcgtcaagtttcgaaattgccgcttgaagatagttcgccaagtctagcgtttcttctagcgcgtgttgcaaccaatcgcgaagcggcaacgggttattgtccgtcgttacgccgtactttgcaagtccaacgattgaacgttgcaacagtaattcgcggttcttttctacgtttttgtcgggcgatttggaagcggcttcgacagcacaacgacaagggccgtttgtgttgtttgtaccgccgccgcatttatgacattcggtcgaatatttcatttgttcaccattcagcggaaagaacttcgggatactttttgttcacccatacgcgaacacggcgcggcgtgcgaagttctgaaacacgctgcaaagcttgataagtcgtcggcggcggttcttcggcgtgccgctgtcgccaccaatcgcgcgaacgtttcgcagcaagccccggatgttcaagcattataaattcgttgaacatttggaagccgcaaaagtaactaaccttaatcatcggcggtttcgttagatttccgtttgcgtcgcgcttttcgtgcaaattgtaaagtaccttttgaacgtcgaaatattcgactatcggcgcgtcgcttcgcagcggttccagcgttccggcagtcgcaaacaacttcgtttcaaaagtaaattcggtgccgcagttaatgcactgtcgggccgcagcgtgattatatacgccgcatacgtcgcaaatacgaacgggcgcgtcgccgccgcctttgcccggtcggttcggaattcgcgggtcgttgatttggccaagccttcgaacgtttccggcgaagtccgcgtacaggcaattttgtttgccagtatccggcgacggtcgggttccgcgtcccaacttttgaacgtgtttgcccggcgatagcgtcgggttcaaatcgccgataaagtcgattggcggatggtcaaaacccgttgtaagtttctgccccgataccaagccgcgaagttcgccagctttgaaagcgcgcaaacgttcggtatttgtcttcgaaggcaacttggaatgaaccggcaaaacttccaagccgtaagactgaattacgttcgcgacgtgttcggtattatcaatgccagttgcgaagataagccaagtcgaacggtcgtaagcaatttcggtcatttcccgaacagcgttaaaaacaacttcgtcggtatctacggcggcttctagttgcttgctgttgaattcgccagccgttacgcctactttcgacaagtcgatttcggttcgcgtcggccttgcgataagcggcgacaagtagccttcggcgataagtcggttaaacgattcgacgccggttatatcgtaacaaatgtcggtaaaaattccgttgtcggtaataagccccattttcattcgatagggcgttgccgtaaatccgataactttaagatgcgggttaatcttgcgaagttcggcgataatgtattggtaatgcgaatcttccttgtcgcttaacaaatggcattcgtcgattaacagcaagtcgcgccaaccgaaatggcgaagatgtgccgggcgtccgtcgtcttcttcaagcccgcgtttaatcgcaggcgctacggactgaacgccgccgaatacgattggcataatcatatcgcgggaattcaagcccgccgaataaatgcccattggcgcggtcggccaaatcgacataagcttttcggcgttctgttcgattagttctttaacatgcgtaagcatcattattcgttgattcggccagtaaccgaaaattcgacgaataaagtttgcaattacgaccgactttccggttcctgtcggcatggcgacgacggggtttccgaccccgccgcgctggaaataatcgaatattgaatattccgcttcgtcttgataccaacgcggaacataaatattagacattctttgcaaccgctgtaattggcgaataagaatcgcaacccgtagcgatgaaatcgcccggaattacgccgttgtgaacttcgcaaaaccattcgccgttttcgacaggatttgcggccttgcagcttcggcagttcttttcaggaatcgcgcccttgtggcaaatatccttagccgcgcaatatccgcacttgtgaaacgtcggattatccgacaagcgcggcggcgcttcctgcgacagaatgatttgttcggccttttccttcatttgctggcctagccgatggtctagctttacaacttcgcaatgcaagtcgtcgtcgttcttgttaatgttcaggtaaagaacataacgaaaacgatattcgttgccatacgtcgaagtttgggcgaaatgttgcggcttgcttactgccattccttgcgacattaagtccgaaaagcctttgccggttccgttggtcttgaattccagcaaaacgggttcgtcgataccgtagcgttcgggaagccgggcgatgccgtcaagcgacccgccgaagtgccccataacgccggaaatgcggtattgtgggaattccaagccgtcggctttcgcgcgtgcgacgtgttgggcgtaatacggattttcgttcgtaataaggtcgcaacccaacggcagttcttcgccttccttcaatatgccgtaactgtcgctttcggcttggtaaaagaagccgtcgcggttttcgtaccaacattgaatgccgatgccttccagccattcgataaagcgggcttcttcacggtgcccacgattaaacaagcgttgcttgcgaccgtccgtcttttcccgaaaacaccaacggaagatataccaaagcttccgcttgcattcgtcgccaatcaaagacgcgccaaggtgccgacggtgcccgccgtcatacgtgcgaacgcaatattcgtctatatcttctttaatgcgcttcgcaagggcggttgcaacgccgggcgcgtcaaggtctacgctttgccttcctgcgtcggatttcgtcggctgcgcgtcgttcagcgttaattgtgcgttcttcgcgtctttgctgtttggcatcgttcttcacctttcgccgcataagggcttcgtaattgttcgctagataatccgccgaaagtgtcgcaacgtctttaagttggtctttcgacagccaagatatatggcattccgacgggtcgattcctaattggttcgcaagccaattgtacgccttcgcgcgcgacattaagccggtttgccaaaggcggtcgaattcgttatgggctttcgttcgaagctggcgcgttgttctgtcggccatacgacccaacggaataaacgtgcccggatggcaaccaacggcggcgcgacaatcattgcaataataaatgtgcggccaattgccataagttcgcccgtaaatcttgtcgttcgttgttagttcaatgttaacagaacaacaagtatcgcattgttcgggcgtcggcaatgcgtcttttattttcgacataaattcgcatactccttaaaaagaaacgccggggccggtcaagaccccggcgaatctacgccgcgacggcgttacgccttaacgctggccccaaggtgccgcgcctgccggtgcgccgccctgcgcgggctggccgccgccctgttgccagccgccgccctgcggttgctgctgcgcgggctgttgggcaggctggccgccccatgccggttggccgccctgcggggccgggttctgcgccggttggccgccccaagctgcgccgccctgcggctgttgggccggttgctgcgcgggctgctgctgtccgccccaagcggcaccgcctgcgggctgctgcggctggccctgcggggcaccgccccaagcgccgttcggctggccctgcggctgctgttgctgcggctgcgctgccgctgcgcctgcgccagccttgcccggttcgttgccgttcatatcgaacacctttttaacttcggtatactgcgggtcgtttttctgcggcccgacttcgataagaaacggcaggttgtgaagctgcgacgaatcggtaacttggaacacgccgattacgtggcagattgccgaaagctggcgatgcgcgatttcgacggtctgttggttggaatggtacaggttcaggcgataagcgccggtcgtgccctgctgcgggccgtcgataatccgcaagttcagttgcagataaccgccgtcgttcgccttgttggccttgacttcggaagattcgacgattaccggatgcttaccaatcggcaggcttccgacgccttgggtcgggtcgtactgttgggcgttgaacgcttggataagttgcatgatgtttcaccttttcgaaaagtcttcgccattggttacggcggcgaagtaaaccgttttattgcatcgctttcgcgaacaatgcggtaaggtcgggctgttcaagttcgttaagattgcccaaacggtcgcgcgcgaaaacttcgggaatttccttcgttcgcagcgcccgaaccggcttcggcattccgggtacgcttgcttcgcccaagtgcataacgttatcgaacaaatgcggaactttaacgttaaggtctttgcccggaaagaacgggcgtttttgcataattggttcgtaagtaacttcgccgttctgcaaaatcgtttgccgtccgttttcgacaagggcttgtttcgcaatcattacgatatgcttttgcggcatgtaatacaagtcgttcgcgattttcattacacgttcggacatattgccgtaagccttcataccgtgtttaaccttgcccaattcgtcggccaagataatttcggcgatattcgaaatactgtcaatacccaacgtatcgaaattcgcagcttcgcgcgatttcataaaccattcgaagaattcgacgataagcgcgggcgaatacgcttcccatgcgggaacgttcgaaccgcgcatggacagcataccgggttcggtcacaagcaaaaccggacgcggcgcagtattgataagcggcgttttgccggaaccgggcgcaccgaatacgacggactttacgccgtagcggcgggccagttgcgacgccggttttaattgcgacatttgcataacttgcaccttcgggaatggccccggcgcttgtgggcaaccggggcggggttgttactttgacttcggcgcgacaagttcaagcgcgggcgttgcttccttcgacgttacaacttcgtcgataagcttacggaacttgtcgggaaggttcttgtattcggtaacggaaagttcgggcttccattttaccaaacgttcggcgataaattcgccttcggggccggtcttttcgattttctgcaaagccttttcgacggcttcttgtccgcctgcgaagctgcggttaatcttgaaaacggctttcagcttgtaacctgcgccaagttcgacgttttcggttccttcgcgcaaagcttcggggtcgaaagcgaaagcgtttttaagaacttcggcgcgcaatgcggattcggcttctttcgctgcggcaagcgccttcgttgcttcctgccattgcagaatcaaagcgtcgcggttagcgttttcgttgaaagacattgttgttactccttcggttgggccgccgcacaattgcgccggtatgtacgaactatacgacggcccttcgttgctgtcaagccccttgttcaagaatttttcgttcttcgaacaagtcgcgattgttggcgtcgaattcggtaaaagcgttcgggaagcgacgacgaagcttcgcgatgttgaccgactgcgcttcgccgaagttcgaaccgatagcacgcagcaaaagggcatcgtaccaaaagccgtcgccgacttcttcaagcgcgttaacagcgtcgaaagcttcgccttcggctgcggcgcttagggcttccaacagttcgcccgcttcggttgccttgccgatgattgcatgaatgatattcacggcggcggcgtcgcggtcgggatggtcggaaatccattcgggaagcttcgccagcgttgccgcgttggcttccggggccggaacgccagtgtcgcgaccgtagaacatggctttcttgattgcgtcaagcttgttaagggcttcgacggcttcggcgatggtttcgcggaagtaggccagcggcacgcggtcgccgtaatacttgtcggacgccgtaacgtgcgcttcttcgatatagtcgaagggctttgcgggttcgttcatacgttcaccttttagaagggccgggcaccatgcgccagcgttccagcactgtaaccgaccgcgcctttcctgtcaacaacaattgacagcaagcaagaagccgggtaagctgcccacaattgctagaaggtggcgttatggacattgaagaacttacgaagcgggtaaagaaagcaagcgtcgggcggtcgctgcgggcgctggccgcgcaatgcaacgtttcgcacgaacttataagaaagcttttgcttgccaattctgcgccgaacataacggcgacgacttataacaagattgataaaggattggcgaagaatggactttaacaatattccgcacgaaatgcggatttacccgcaatgggtcgtttggcgatacgaagacacggattcaaagaaaccgacgaaggttccgtattcagcaaaaaccgggcaccttgccagcgtaaccgacccgaacacttgggccgggttcgacgaatgcgttaacgctatgtcgtccggttggtatgccggaatcggtttcgtattgactgaaaacgacccgtattcgtttatcgaccttgacgacacaaaaggcgaccaaacggcgcttgaccgccaaataaagatttttaacgaattcaacagctacgccgaacggtcgccttccggttcggggttgcatatcatcgttaagggcgcgattccgtcgggccgccgtcgttcgtttatcgaagtttattcttcgcttcgttatatgacaatgaccggcgatatttaccgtaacgcgccgattaacgattgcaacgaactattaaacgttctttggggccaaatggggcaaggttcggtcgccgttgcgcattatgccggacttgccgaagccaaggaaaccgacgaacaggtttataaccgcgcagtcgccgcagccaatggcgacaagttcgccgaactgtacgcgggcaaatgggaaggcatgtacgcttcgcagtccgaagccgactttgccttggtcgatattatcgcgttttatacgcagaaccgggcgcagatttcgcgaatgtttcgcgcgtcgggcttggggcagcgtgacaaagcaaaacgcgacgattacgtttcgtacatgctgaacaagtgtttcgaccgcatgttgccgcccgttgacgttgacggattgcgcaacaagctagacgaagcaatagcaaagaaagaagccgccgacagggccgccgcgttgtcgcagaacagcgaagcgacgccgcatccgaaagccccggccccgaaccttaacgaagcttcgaaggtatacagcgtgccgcccggattagtcggagaaatcgcgcaatacatttacgcacaagcgccgcgcccggtgcccgaaatcgcgttggccggtgcccttggcttggtcgccggtattgtgggcagggcgtacaacatttccggcactggccttaatcaatacgttctgttgttggcaccgaccggaacaggtaaagaagccatcgcaagcggcattgataagctaatggcgcaggttatccgaaccgttcccgccgcgtcggactttatcggccccggcgaaattgcttcgtcgcaagcgattattaagtatatgtcgcgcgggccaacgtcgttcgtttcgttggttggcgaatttggcatttatcttcaacaaatggcaagcgtcaacgcaccgccgcaccttatcgggcttcgtcgcttcctgttggatgcttacaacaagtcgggcgaaggcaaggtacttcggccttcgatttattcagacaaggacaagaacaccgccgcagtattggccccgtcttttaccttgcttggcgaatcgacgcccgaaaagttttacgaaggcttgcacgaaggtttgatttccgaaggtctgttgccgcgttttacgatgattgaatatcacggcgaacgcccggcgttgaatccggggcacctgtcggcccaaccttcgttcgaacttatcgacaggctttcgaccttgtgcgcccatgcgctaatgctgaacagccaacataaggcgatacacgttcaaaccgacgcaaccgcccgcgaactgttccagcaattcgacgcgcattgcgacgcgaacattaacacaagcgaccgcgaagttcggcggcacctttggaaccgggcgcacgtaaaggcgttgaagctggccggaattatcgccgttggctgcaacccttacgacccaaccattaccgccgacgttgcgtcttgggcgattaaccttgtcgtcgccgacgttcgaaacttgcttgcccggttcgatgctggcgaaattggcatagacaacgacgaaacgaaacagcttgcgaaggttattgcaaccgttaaagatttcgtcgtttcaccttggccggacgttgcgaagtacgcaggcgaaggaatgtccaaccttcattcgaaccgaattgttccgtacagctacgttcaacgcaggcttgccgctgttgccgtctttcgtaaagaccgcatcggcgcaagcggggcaatcaagcgcgccttgaagaccctttgcgaacgcggcgatttgcaggaagtaagccgggccacactggcgaaggattacggaacaagcgccgttgcatacatggtcgcgcatccgggcgttttcggcctgtaacgcgcgcccgccagtgtgggcagaacgggccgccttcgggcggctttttcgtgcctgtaaaaaagttcgtcgtacctattgacgaagcttcgaagttgccgtatatttgaaccatcgaagcaaacaacgaaggattaacgaacatgaacgcacttaacaacattcaacgggtcgtaagctggaacagcaagaagaacgacgacggcacctttaccgctaccgcgtacagcttcgaccataacgcgccgaccgtcgtacatgccagctacacgcgcgccagccgcgcccaagccgtcgcagacgccaagaaggccgttcgttacctgaaagcccaacagcgcaccgcgtaaggagtcgccgccatgtttgcccattacttcgccagcaagaaaacgaagttcgttgtaatcagcgaaacgaaccgcccggaaggccagcgaatcgccgtaagcggcaaagccgaagcccgcagggtcgccaaggaacgcaacgcgcagccttggaacttctaaccccggccccggcccttggcacgcgctaggggccgcgcagcctgcccacaatcaacggaagccgcagccatgacccgacagcccttcacaaacgcaaccatgcgcgaaccgacgcccggtaagccgcacattgccctaattgccggatggtggcgcgtgtcgccttggaagcgcggaaccggggcgtcgtactatcaagcgcacgcattcgtaaacaagttgaacagacaaaggagtttgaacaaatgaccgcatattttatcgcatttggcgtcgcgcttgggttggcccttgcgcgcttggccgcttcccaattcgaagccgcttattacctgttctgcaacggcgaatttcgaaaggcattccgggcaacgatgcgcgcccttacctgcgttgcgttgcttgcgttggttgtttcgcccgttgcttcgttcttcgatagcttcgaagttataagcattgaacaagcttcgcccaatccttcgaagggtcttcgcgtataatagccgacgggtcgtataatggcccgtcataacgcttaaacccttgatacacaaggcttttaacggatttatagcaagtataacgtttaaggccgttccacctgtaccggggcgcactctttattaaaagtcactattgattaatagtaatatttttactattatattgtattatattattatatttcctttattttcaaggacttagcagctatacgacccgttcaatccgtataatgctttatcaattgattaattgttgacacttgataaaaagtaagctaggcttgcactattgattaaggggcttgctatgccgaaaccaacgacgaagaagggccgaccaaagggctttattccgaagcctgcgaactgcggccagtgtttgcgcgaagtagcgccgaacatgaaaatttgtccgtattgcttgaagtcaaccgggcttgtatcgactgcgaaggagttaaagaaatgaccgaagaaacgaagaaggttcaaattttaccgtcgtcgccgaaggcgcttgccttgtgcgaagtttcgacggacaatcaaccggaacgcacgccggacgaagacaacgcgaaatatccgtttcgttcgctgcaagtcggcgaatcgttcgcgataccgtttgcagatacgaaccccggaacgcttgcgtcgcttcgttcgtcggccagttcatacggcaagcggcttaaccgcaagtatcgcgttttcgttcacgacgaatataagtgcgtcgaagttgcgcggctgaaatgaacggcaacgcgcggcccaatgtgggcaagccggttcgcgtgtatgggtcgtcgtatcttggccttcgcgcgcagtacccgaacgcctttgccatccaaccaacccggacgggctttcaagccgtcgtaatcattgaagaaggggcgaagcatgtacgaaatcgaaaccggccataaagtgccgaagcaacgccgcaaggctggaagcgtgccgaaggccgttcaacaggcgttcaacgactacgccgacgcatataaggccgtttacggcgttcgaccgctgtcgttcacgtatgacagcgaaagcggctttattcgtgtcgaaagtagcggcggcgtaagcgtcgcaaggctgcgcgaaatgacgaaacaacttcgttaccgcaaaggctgaaaaaagttgttcgcaggtattgacgaagcgtcgaaggcgtcgtactatagacccataccaacgaacacaaggaaccgccgaaatgaacgtaaccaaccttaaaaccgccgtcgaaatcaaaattgaaatcgaattggccgcttgggccaacggcgaaaagaaagttaacgtttccaaccaattcgacgaaagcgttttggaatcggcgaaagaagcaatttccgtcgaagcaatcgccgcaatcgttgccaagtatccgggcgcgaacttcgaaggcttttcggttatgacttgggcgcacgaactttcggctttcaaagccccggaaatcgaccgcgcttggttcgattaatcaacagcgcgccgggcgcaacccggcatttttgaaggagttacaacaatgtgcatcgtatgtgatattaaacaggccgtcgaagcttccggcccgaacaaagaagaccgcgccaaaatccttggcttggtcgaaaagctggccgaagctttgggcgatgttctggaagtcgcgcaggaagtacacgaagccaagcccgaagcgttccagccggaacacgtcgaacgcttgcagaacgccgccgacttgctgaacgaccggggcgaactgcccgacgccctgttggccctgctgttggccgcccttgggcgcggcgtcaaggtcgaaacaatccgcgttgaactgcgcgaaggcgaaacgccagaacaggccgtagcgcgtgtaatggccgaacgcgaaagcggggccgcgacgaaacactaaccaaagcgccccggctgttgtatagtcggggcttctttctatcatggggaacgaaagaacatggcggacgaagtagaccaaacagccgaccgaatagaaaacgaagtaagctttacggtcggcgaactttgccgaaaggccgcagcgatacccgcaggccgtccgggcgaatgtgatttttgcggcgaacacttcgcgcgcgttgtcgaagtgaccgacccgcgaacgggcgaagtcgtcgaaagctgcggtcgctgtcgtgaccgaaggggcatcgcatgacgcccgcaacccttgctaagtctggcaccgaacacggccaccaagcggcgttattcgcttactgcgccgtcgcgtatcttcacggcttcgacgtagccgacgaatggtgcaagaccggcgtaatcccgcaaacgacgccgtacagcatgtacgaaacgccgaccgtgcccgcgcttgaatggttccacgctatccacaaccaaggccacggcgacaaggtgcgcggggctaacgccaaggccgaaggcgtccgcaagggcgtagccgatacgttcttgccttggccgaatggcggatggcatggcctttatatcgaaatgaagaagccgaccgaacgcccgaagtcggaaaccgcaaagggcggcgtatcggacgaacaacgaagattcggcgaatatgcaaagcgcgtcggctatggttgggccgtctgctatggttgggaacacgccgtaacgacgttgcgaagttatatcgaatggggttcgtaatggggctttcgtgccttgcctgcgaacttacccgcgcccggttgaaagcggcggcgctggcccttgtgggctggccccttgaccgcatcgccgggcatttgtccgtttgctatggcgaacggtattacgtcgaaggcggcaagctgtatcgcgcgtcgaagttgccgccgtatcaaccgcacttgataaggggcgaacaatgaaaaagaccgacgaagaattgatagacgaagcccgcagcattgcgcgttcgaaacgctgtttcgtcgtaacgaagccgggttattggctgctgtaccgcgaatcggtgccgcgtaacgtatgcgtcggcaccgggttattggctgctgtaccgcgaatcggtgccgcgtaacgtatgcgtcggcaaacggtcgtcggcttcggcgttgttgcaacttgcgaaaaaggcttgacgcagcttcgaagctgtcgtacacttcttcgtaagttgaacgaatcaaggagtaacgacaatgcccgcatataacgtaacaactgaattcgaaatgaccgacggtcgcgttctgtcgtgcgaatacggcgtatcgtatacgcccgcttacattagcggcccgcccgaagactgttacccggaagaaagcgacgcgggcgaaccgacgtactttatcgacggcgaagaagtcgattataaagaccttccaaaaggcttggacgaaatcgccgacaagctttacgaagcggggccgggcgaatattcgtattcgcaatcggacgttgacaacgaaccggattacgaaccggattacgattactattaacgaaggagtaacgaaaatgtcttggcttatcggttggggcgtactttccgtcggcgtaatcgtcggcttcttccttgcggccttgctgcgggccaatgggcgcgacgtgccggttccttcggctaccgttaccgccctgtcgccgcaggaacgcgcccgcatgggctacgcgctggcaagggctggcgacttgctggacagcggcgaccttgaatacgtgtcgggcggctttatggtgcaagacgtaggacacggcgtcgtaattataaaaggcgatttgtcgttgcgggttgccgaagatgaataaggacgaagcgcgcgaaatgttcgaagccgtcaaggccaaccgggcgaagattgacggttgcgcccgccatcgcttcgaaattggcgacccgccgtacacgttcgggcaaaagttcacttgttcgaactgcggcggaacaatggacgccgtacaggcgttccgatactgtcaaggcttcaaggccgcaggcggcgacccgaacgaagttataccgggttacgaataacgcttgacaagcggcgaaggttcgacgaaacttagcacgtacccaacaaaggagttacgaacatgaatttcgacccgctgtttcttaccatcggactttcggcgcttgcttgcgcttgttacttgaagttcggccaaatcaaagcgaagcgcgaacaagaacgccgcattcgcgaagccatcgaacgcgcgcaggttgtgaaggcacgcggcgaaattcgcggcaagaagcttgccaacgaacgcgaatggggcttggcggaagattacaaccccggtaagttctggccgcagtaatggcgataatctacgcaccgcgcgaagccctttcaaaatgggacgcgcgatttattgaactggccgaacacgtcgccggatggtcgaaagggccgcgtaagcgcgtcggcgcggctatcgttcgcccgaatcggtctattgcgtcgcttgggtacaacggcccgccgcgcggcttcgacgacggcgtttttctgaacatgacgcgcgacgaacaacacgcggtcgcaattcatgccgaagacaacgcaattcgacaggctgcgccgggcgaagacttgtccgcgtgtacgctgtacgtttcgccgctgtttccgtgcgccatttgtgccgaccgcatcgttcgggccggtatccgtcgcgttgtcgcttattgtgggcatatatcgccagactggcgcgcgtctgccgacgaagccgaacgcatctttaaccaagcgggcgtcgaatgcctgtttacaatggattaacgaacatgaagccgctagaccattcgcaaatcgaagcgttgttgttctatcaagacccgacgacgcaaaattatatcggcgcaccgaaggccgacccgttcaaccaagccggaagctttgtcgcattcgggccgcgtgttaccgttgacccggcgttgtataacttgcttgccgcagcgccgacaatgtaccaagccctttcgatgcaatacgcttaccttcaagcgcaaatcgaagttatcgaacgcttgccaaaggcgggcgaacttgataagctgttgtcgtcgttaatcgaagcgcagaacgcttgtctaatggcccaacgtatcgcgcaagtcggttacgaaaatgtcgcaaattcacttgacaaaggttcgaagcggtcgtaagcttgaaccatcgaaacgaacaaaggtgcccacaatgaaccgtaagcttcttgttatcgctggaatcgtcgccttcgtcgcgttgcttggtatggccgggcaaatggacttcgaagacgaagcccgcgcgcacctgttgtattgtgacaacgtagcgaacggcgtttggccggattacgacaaaatttacgattcggaatgcacgcccgaacgcatcgcagaaatcgaagaaattttgcgttgaccgcttgacacgaagaacggtcggcgtaaaatcaacccgtcgcaacaacgcgacataaccttaacgttaaggagttacacaaaatggctaccaagaaatcgaccgcgaagaagaacaccgccgccccggttatcggccttgccgaaattgttgcagccgggccgaatggtctgtatacttcgcctgccgtacatggcccgcttgtcgaagccggtatggtggaaatcaacccggcaatgaccaacgaagcgggcgaaatcgcaacccgcgcaacccaaaaaggaatcgaagaaatgaaccagaacaccgaaaccggcaccgccgcagcttccgccccggtcgctacttccttcaccatcgaagacaacgtaccgatgccgaccggcagcggtcgcggtcgcggcggcaacgtctacccgttcgacgcgctggaagtcggccaaagcttcttcgttccgaacagcgaagaaaagccgaacgccgcgaagtcgcttgcttcgaccgtttccagcgcaaccgcccgtttcgccgtgccttccgaagacggcgcgaccaagaccaacaagaagggcgaaaccgtgcccgttatggtcgaaacccgcaagttcgttgttcgttcggtcgaaggcggcgcgcgggtctggcgtaccaagtaagcgacggcgcgggctacggcccgccctacgcctacgcttcaacggaaaccccggccattgcgccggggttttcttttgcctttcttgtcaatttgtgctaatccgtgctaatcttcggccaaatacatttcggggccggggcttgtgaatgaacgaacaacaattttttaacgtagctgtcgcaattatcggcgcgttgggcggttggtggatgcgcgttatgtggcagtcacttaaagaacttcaagcgcaagattcgaagttggccgataaagtcggcaatatcgaagttcttgtagccggacagtacgtcaagcgcgacgatatgaaccgcgacataatggcgattttcgccaaacttgaccgcatcgaagacaagatagacaaaaaggccgacaaatgaagaagcccgaacttatcgaagattggcgcaattggtggcgcttttggtcggttcgactggccgcagtcggcaccgcaattactggccttcttgttgcgtttcccgacgcagctttggccgcttgggcaatccttccgcacgaattgaagtcgtcgattccgccgcagtatatgccgcttatcggcgttgttgttttcgcgctttccatcgttgcccgccttgtcaagcaaaagaccttgaacaaggggccgaccgatgaataacgaacttccttgggtagccgaagcccgaaagtatatcggccttcgcgaagacacttcgaagacttcgcataacccgaagcttcttgccatgcttgaccgcatgggcgaattttccaacgaatcccgcgcttggtggcacgacgacgaaacgccttggtgcggactgttcgtcggctattgcttgggcgtagccgggcgctacgtcgtccgcgaatggtacagggcgcgggcatgggaagccccgcagcttacgaagcttgaccggcccgcatacggcgcgcttgtgaccttcacgcgaagcggcggcggccacgtcggttttattgtgggcaaggatgcgcgcggaaatcttatggttcttggcggtaatcagtcgaacgccgtaagtattgcaccgttcgcagtatcccgcgtaaccggctatttctggccgtcgttctggcgaaacaagaccgcagttaaaagcgttccgtttgaagaacgttattcgctgccgctgttgaagtcgaacggcgaactttcgacgaatgaagcgtaaaggggcatcgtatgttttccgtaatttgggccaagtttggcaaatggcttgccgcaatcggcgcgggtcttgtcatgctggcaagtattttttatgccggtcgcaagtccggcgcaaccaaggccgaagccaacgcagcaaacgaacgggcaaacgaccgcgaagcaatcgcagttcgccaagttaacgaagcccgcgaagcttccgaacaacaggtaaaggcggtacaaaatgcgaaagacgttgcttccgataattctacttttgacgacgacgaagttactaagcggctgcgcgacgaatggtcgcgcgactgaaccgcaaagcatcgccgacgcagtgcaaacgaagcccgttgtaatcgacacggcttgcaaatgggtttcgcccatttggatttcgaaggccgacggcttgaccgctggcacggcccggcaaattctgaaccataacgaagccgtcgaacgcaattgcgggccgcagtcgccgcctaaatctgcggacaagccttaacagaa